European Patent Specification EP 3 868 779 B1, published November 6, 2024. Title: COMPOSITION BASED ON RECOMBINANT BIOPOLYMERS AND USES OF THE SAME AS BIO-INK. Applicant: Universidad de Valladolid. The sequence listing filed with the application follows.

SEQUENCE LISTING (29 sequences)

SEQ ID NO: 1 - DNA, 18 bp, Artificial Sequence
  Additional 5´ sequence
atggaatccctgctgccg

SEQ ID NO: 2 - protein, 25 aa, Artificial Sequence
  Monomer B
VPGVGVPGVGVPGEGVPGVGVPGVG

SEQ ID NO: 3 - protein, 5 aa, Artificial Sequence
  Monomer C
VGIPG

SEQ ID NO: 4 - protein, 53 aa, Artificial Sequence
  Monomer X: zipper structural domain
VGGGGGKENQIAIRASFLEKENSALRQEVADLRKELGKCKNILAKYEAGGGGG

SEQ ID NO: 5 - protein, 32 aa, Artificial Sequence
  Monomer Y: silk structural domain
VGAGAGSGAGAGSGAGAGSGAGAGSGAGAGSG

SEQ ID NO: 6 - protein, 223 aa, Artificial Sequence
  Monomer D: comprises cell adhesion protein motifs or peptides
VPGIGVPGIGVPGIGVPGIGVPGIGAVTGRGDSPASSVPGIGVPGIGVPGIGVPGIGVPGIGAVTGRGDSPASSVPGIGVPGIGVPGIGVPGIGVPGIGAVTGRGDSPASSVPGIGVPGIGVPGIGVPGIGVPGIGAVTGRGDSPASSVPGIGVPGIGVPGIGVPGIGVPGIGAVTGRGDSPASSVPGIGVPGIGVPGIGVPGIGVPGIGAVTGRGDSPASSV

SEQ ID NO: 7 - protein, 5 aa, Artificial Sequence
  ELR domain
  MISC_FEATURE (4)..(4): Xaa is selected from any natural amino acid except proline
VPGXG

SEQ ID NO: 8 - protein, 6 aa, Artificial Sequence
  Region of the silk protein sequence
GAGAGS

SEQ ID NO: 9 - protein, 3 aa, Artificial Sequence
  RGD domain
RGD

SEQ ID NO: 10 - protein, 4 aa, Artificial Sequence
  REDV domain
REDV

SEQ ID NO: 11 - protein, 1329 aa, Artificial Sequence
  Protein sequence of the biopolymer 1
MESLLPVPGVGVPGVGVPGEGVPGVGVPGVGVPGVGVPGVGVPGEGVPGVGVPGVGVPGVGVPGVGVPGEGVPGVGVPGVGVPGVGVPGVGVPGEGVPGVGVPGVGVPGVGVPGVGVPGEGVPGVGVPGVGVPGVGVPGVGVPGEGVPGVGVPGVGVPGVGVPGVGVPGEGVPGVGVPGVGVPGVGVPGVGVPGEGVPGVGVPGVGVPGVGVPGVGVPGEGVPGVGVPGVGVPGVGVPGVGVPGEGVPGVGVPGVGVGIPGVGIPGVGIPGVGIPGVGIPGVGIPGVGIPGVGIPGVGIPGVGIPGVGIPGVGIPGVGIPGVGIPGVGIPGVGIPGVGIPGVGIPGVGIPGVGIPGVGIPGVGIPGVGIPGVGIPGVGIPGVGIPGVGIPGVGIPGVGIPGVGIPGVGIPGVGIPGVGIPGVGIPGVGIPGVGIPGVGIPGVGIPGVGIPGVGIPGVGIPGVGIPGVGIPGVGIPGVGIPGVGIPGVGIPGVGIPGVGIPGVGIPGVGIPGVGIPGVGIPGVGIPGVGIPGVGIPGVGIPGVGIPGVGIPGVGIPGVPGVGVPGVGVPGEGVPGVGVPGVGVPGVGVPGVGVPGEGVPGVGVPGVGVPGVGVPGVGVPGEGVPGVGVPGVGVPGVGVPGVGVPGEGVPGVGVPGVGVPGVGVPGVGVPGEGVPGVGVPGVGVPGVGVPGVGVPGEGVPGVGVPGVGVPGVGVPGVGVPGEGVPGVGVPGVGVPGVGVPGVGVPGEGVPGVGVPGVGVPGVGVPGVGVPGEGVPGVGVPGVGVPGVGVPGVGVPGEGVPGVGVPGVGVGIPGVGIPGVGIPGVGIPGVGIPGVGIPGVGIPGVGIPGVGIPGVGIPGVGIPGVGIPGVGIPGVGIPGVGIPGVGIPGVGIPGVGIPGVGIPGVGIPGVGIPGVGIPGVGIPGVGIPGVGIPGVGIPGVGIPGVGIPGVGIPGVGIPGVGIPGVGIPGVGIPGVGIPGVGIPGVGIPGVGIPGVGIPGVGIPGVGIPGVGIPGVGIPGVGIPGVGIPGVGIPGVGIPGVGIPGVGIPGVGIPGVGIPGVGIPGVGIPGVGIPGVGIPGVGIPGVGIPGVGIPGVGIPGVGIPGVGIPGVPGIGVPGIGVPGIGVPGIGVPGIGAVTGRGDSPASSVPGIGVPGIGVPGIGVPGIGVPGIGAVTGRGDSPASSVPGIGVPGIGVPGIGVPGIGVPGIGAVTGRGDSPASSVPGIGVPGIGVPGIGVPGIGVPGIGAVTGRGDSPASSVPGIGVPGIGVPGIGVPGIGVPGIGAVTGRGDSPASSVPGIGVPGIGVPGIGVPGIGVPGIGAVTGRGDSPASSV

SEQ ID NO: 12 - protein, 1233 aa, Artificial Sequence
  Protein sequence of the biopolymer 2
MESLLPVPGVGVPGVGVPGEGVPGVGVPGVGVPGVGVPGVGVPGEGVPGVGVPGVGVPGVGVPGVGVPGEGVPGVGVPGVGVPGVGVPGVGVPGEGVPGVGVPGVGVPGVGVPGVGVPGEGVPGVGVPGVGVPGVGVPGVGVPGEGVPGVGVPGVGVPGVGVPGVGVPGEGVPGVGVPGVGVPGVGVPGVGVPGEGVPGVGVPGVGVPGVGVPGVGVPGEGVPGVGVPGVGVPGVGVPGVGVPGEGVPGVGVPGVGVGIPGVGIPGVGIPGVGIPGVGIPGVGIPGVGIPGVGIPGVGIPGVGIPGVGIPGVGIPGVGIPGVGIPGVGIPGVGIPGVGIPGVGIPGVGIPGVGIPGVGIPGVGIPGVGIPGVGIPGVGIPGVGIPGVGIPGVGIPGVGIPGVGIPGVGIPGVGIPGVGIPGVGIPGVGIPGVGIPGVGIPGVGIPGVGIPGVGIPGVGIPGVGIPGVGIPGVGIPGVGIPGVGIPGVGIPGVGIPGVGIPGVGIPGVGIPGVGIPGVGIPGVGIPGVGIPGVGIPGVGIPGVGIPGVGIPGVGIPGVGAGAGSGAGAGSGAGAGSGAGAGSGAGAGSGVGAGAGSGAGAGSGAGAGSGAGAGSGAGAGSVPGVGVPGVGVPGEGVPGVGVPGVGVPGVGVPGVGVPGEGVPGVGVPGVGVPGVGVPGVGVPGEGVPGVGVPGVGVPGVGVPGVGVPGEGVPGVGVPGVGVPGVGVPGVGVPGEGVPGVGVPGVGVPGVGVPGVGVPGEGVPGVGVPGVGVPGVGVPGVGVPGEGVPGVGVPGVGVPGVGVPGVGVPGEGVPGVGVPGVGVPGVGVPGVGVPGEGVPGVGVPGVGVPGVGVPGVGVPGEGVPGVGVPGVGVGIPGVGIPGVGIPGVGIPGVGIPGVGIPGVGIPGVGIPGVGIPGVGIPGVGIPGVGIPGVGIPGVGIPGVGIPGVGIPGVGIPGVGIPGVGIPGVGIPGVGIPGVGIPGVGIPGVGIPGVGIPGVGIPGVGIPGVGIPGVGIPGVGIPGVGIPGVGIPGVGIPGVGIPGVGIPGVGIPGVGIPGVGIPGVGIPGVGIPGVGIPGVGIPGVGIPGVGIPGVGIPGVGIPGVGIPGVGIPGVGIPGVGIPGVGIPGVGIPGVGIPGVGIPGVGIPGVGIPGVGIPGVGIPGVGIPGVGIPGVGAGAGSGAGAGSGAGAGSGAGAGSGAGAGSGVGAGAGSGAGAGSGAGAGSGAGAGSGAGAGSV

SEQ ID NO: 13 - protein, 1213 aa, Artificial Sequence
  Protein sequence of the biopolymer 3
MESLLPVPGVGVPGVGVPGEGVPGVGVPGVGVPGVGVPGVGVPGEGVPGVGVPGVGVPGVGVPGVGVPGEGVPGVGVPGVGVPGVGVPGVGVPGEGVPGVGVPGVGVPGVGVPGVGVPGEGVPGVGVPGVGVPGVGVPGVGVPGEGVPGVGVPGVGVPGVGVPGVGVPGEGVPGVGVPGVGVPGVGVPGVGVPGEGVPGVGVPGVGVPGVGVPGVGVPGEGVPGVGVPGVGVPGVGVPGVGVPGEGVPGVGVPGVGVGIPGVGIPGVGIPGVGIPGVGIPGVGIPGVGIPGVGIPGVGIPGVGIPGVGIPGVGIPGVGIPGVGIPGVGIPGVGIPGVGIPGVGIPGVGIPGVGIPGVGIPGVGIPGVGIPGVGIPGVGIPGVGIPGVGIPGVGIPGVGIPGVGIPGVGIPGVGIPGVGIPGVGIPGVGIPGVGIPGVGIPGVGIPGVGIPGVGIPGVGIPGVGIPGVGIPGVGIPGVGIPGVGIPGVGIPGVGIPGVGIPGVGIPGVGIPGVGIPGVGIPGVGIPGVGIPGVGIPGVGIPGVGIPGVGIPGVGIPGVGGGGGKENQIAIRASFLEKENSALRQEVADLRKELGKCKNILAKYEAGGGGGVPGVGVPGVGVPGEGVPGVGVPGVGVPGVGVPGVGVPGEGVPGVGVPGVGVPGVGVPGVGVPGEGVPGVGVPGVGVPGVGVPGVGVPGEGVPGVGVPGVGVPGVGVPGVGVPGEGVPGVGVPGVGVPGVGVPGVGVPGEGVPGVGVPGVGVPGVGVPGVGVPGEGVPGVGVPGVGVPGVGVPGVGVPGEGVPGVGVPGVGVPGVGVPGVGVPGEGVPGVGVPGVGVPGVGVPGVGVPGEGVPGVGVPGVGVGIPGVGIPGVGIPGVGIPGVGIPGVGIPGVGIPGVGIPGVGIPGVGIPGVGIPGVGIPGVGIPGVGIPGVGIPGVGIPGVGIPGVGIPGVGIPGVGIPGVGIPGVGIPGVGIPGVGIPGVGIPGVGIPGVGIPGVGIPGVGIPGVGIPGVGIPGVGIPGVGIPGVGIPGVGIPGVGIPGVGIPGVGIPGVGIPGVGIPGVGIPGVGIPGVGIPGVGIPGVGIPGVGIPGVGIPGVGIPGVGIPGVGIPGVGIPGVGIPGVGIPGVGIPGVGIPGVGIPGVGIPGVGIPGVGIPGVGIPGVGGGGGKENQIAIRASFLEKENSALRQEVADLRKELGKCKNILAKYEAGGGGGV

SEQ ID NO: 14 - protein, 1435 aa, Artificial Sequence
  Protein sequence of the biopolymer 4
MESLLPVPGVGVPGVGVPGEGVPGVGVPGVGVPGVGVPGVGVPGEGVPGVGVPGVGVPGVGVPGVGVPGEGVPGVGVPGVGVPGVGVPGVGVPGEGVPGVGVPGVGVPGVGVPGVGVPGEGVPGVGVPGVGVPGVGVPGVGVPGEGVPGVGVPGVGVPGVGVPGVGVPGEGVPGVGVPGVGVPGVGVPGVGVPGEGVPGVGVPGVGVPGVGVPGVGVPGEGVPGVGVPGVGVPGVGVPGVGVPGEGVPGVGVPGVGVGIPGVGIPGVGIPGVGIPGVGIPGVGIPGVGIPGVGIPGVGIPGVGIPGVGIPGVGIPGVGIPGVGIPGVGIPGVGIPGVGIPGVGIPGVGIPGVGIPGVGIPGVGIPGVGIPGVGIPGVGIPGVGIPGVGIPGVGIPGVGIPGVGIPGVGIPGVGIPGVGIPGVGIPGVGIPGVGIPGVGIPGVGIPGVGIPGVGIPGVGIPGVGIPGVGIPGVGIPGVGIPGVGIPGVGIPGVGIPGVGIPGVGIPGVGIPGVGIPGVGIPGVGIPGVGIPGVGIPGVGIPGVGIPGVGIPGVGIPGVGGGGGKENQIAIRASFLEKENSALRQEVADLRKELGKCKNILAKYEAGGGGGVPGVGVPGVGVPGEGVPGVGVPGVGVPGVGVPGVGVPGEGVPGVGVPGVGVPGVGVPGVGVPGEGVPGVGVPGVGVPGVGVPGVGVPGEGVPGVGVPGVGVPGVGVPGVGVPGEGVPGVGVPGVGVPGVGVPGVGVPGEGVPGVGVPGVGVPGVGVPGVGVPGEGVPGVGVPGVGVPGVGVPGVGVPGEGVPGVGVPGVGVPGVGVPGVGVPGEGVPGVGVPGVGVPGVGVPGVGVPGEGVPGVGVPGVGVGIPGVGIPGVGIPGVGIPGVGIPGVGIPGVGIPGVGIPGVGIPGVGIPGVGIPGVGIPGVGIPGVGIPGVGIPGVGIPGVGIPGVGIPGVGIPGVGIPGVGIPGVGIPGVGIPGVGIPGVGIPGVGIPGVGIPGVGIPGVGIPGVGIPGVGIPGVGIPGVGIPGVGIPGVGIPGVGIPGVGIPGVGIPGVGIPGVGIPGVGIPGVGIPGVGIPGVGIPGVGIPGVGIPGVGIPGVGIPGVGIPGVGIPGVGIPGVGIPGVGIPGVGIPGVGIPGVGIPGVGIPGVGIPGVGIPGVGIPGVGGGGGKENQIAIRASFLEKENSALRQEVADLRKELGKCKNILAKYEAGGGGGVPGIGVPGIGVPGIGVPGIGVPGIGAVTGRGDSPASSVPGIGVPGIGVPGIGVPGIGVPGIGAVTGRGDSPASSVPGIGVPGIGVPGIGVPGIGVPGIGAVTGRGDSPASSVPGIGVPGIGVPGIGVPGIGVPGIGAVTGRGDSPASSVPGIGVPGIGVPGIGVPGIGVPGIGAVTGRGDSPASSVPGIGVPGIGVPGIGVPGIGVPGIGAVTGRGDSPASSV

SEQ ID NO: 15 - protein, 1455 aa, Artificial Sequence
  Protein sequence of the biopolymer 5
MESLLPVPGVGVPGVGVPGEGVPGVGVPGVGVPGVGVPGVGVPGEGVPGVGVPGVGVPGVGVPGVGVPGEGVPGVGVPGVGVPGVGVPGVGVPGEGVPGVGVPGVGVPGVGVPGVGVPGEGVPGVGVPGVGVPGVGVPGVGVPGEGVPGVGVPGVGVPGVGVPGVGVPGEGVPGVGVPGVGVPGVGVPGVGVPGEGVPGVGVPGVGVPGVGVPGVGVPGEGVPGVGVPGVGVPGVGVPGVGVPGEGVPGVGVPGVGVGIPGVGIPGVGIPGVGIPGVGIPGVGIPGVGIPGVGIPGVGIPGVGIPGVGIPGVGIPGVGIPGVGIPGVGIPGVGIPGVGIPGVGIPGVGIPGVGIPGVGIPGVGIPGVGIPGVGIPGVGIPGVGIPGVGIPGVGIPGVGIPGVGIPGVGIPGVGIPGVGIPGVGIPGVGIPGVGIPGVGIPGVGIPGVGIPGVGIPGVGIPGVGIPGVGIPGVGIPGVGIPGVGIPGVGIPGVGIPGVGIPGVGIPGVGIPGVGIPGVGIPGVGIPGVGIPGVGIPGVGIPGVGIPGVGIPGVGIPGVGAGAGSGAGAGSGAGAGSGAGAGSGAGAGSGVGAGAGSGAGAGSGAGAGSGAGAGSGAGAGSVPGVGVPGVGVPGEGVPGVGVPGVGVPGVGVPGVGVPGEGVPGVGVPGVGVPGVGVPGVGVPGEGVPGVGVPGVGVPGVGVPGVGVPGEGVPGVGVPGVGVPGVGVPGVGVPGEGVPGVGVPGVGVPGVGVPGVGVPGEGVPGVGVPGVGVPGVGVPGVGVPGEGVPGVGVPGVGVPGVGVPGVGVPGEGVPGVGVPGVGVPGVGVPGVGVPGEGVPGVGVPGVGVPGVGVPGVGVPGEGVPGVGVPGVGVGIPGVGIPGVGIPGVGIPGVGIPGVGIPGVGIPGVGIPGVGIPGVGIPGVGIPGVGIPGVGIPGVGIPGVGIPGVGIPGVGIPGVGIPGVGIPGVGIPGVGIPGVGIPGVGIPGVGIPGVGIPGVGIPGVGIPGVGIPGVGIPGVGIPGVGIPGVGIPGVGIPGVGIPGVGIPGVGIPGVGIPGVGIPGVGIPGVGIPGVGIPGVGIPGVGIPGVGIPGVGIPGVGIPGVGIPGVGIPGVGIPGVGIPGVGIPGVGIPGVGIPGVGIPGVGIPGVGIPGVGIPGVGIPGVGIPGVGIPGVGAGAGSGAGAGSGAGAGSGAGAGSGAGAGSGVGAGAGSGAGAGSGAGAGSGAGAGSGAGAGSVPGIGVPGIGVPGIGVPGIGVPGIGAVTGRGDSPASSVPGIGVPGIGVPGIGVPGIGVPGIGAVTGRGDSPASSVPGIGVPGIGVPGIGVPGIGVPGIGAVTGRGDSPASSVPGIGVPGIGVPGIGVPGIGVPGIGAVTGRGDSPASSVPGIGVPGIGVPGIGVPGIGVPGIGAVTGRGDSPASSVPGIGVPGIGVPGIGVPGIGVPGIGAVTGRGDSPASSV

SEQ ID NO: 16 - protein, 1508 aa, Artificial Sequence
  Protein sequence of the biopolymer 6
MESLLPVGGGGGKENQIAIRASFLEKENSALRQEVADLRKELGKCKNILAKYEAGGGGGVPGVGVPGVGVPGEGVPGVGVPGVGVPGVGVPGVGVPGEGVPGVGVPGVGVPGVGVPGVGVPGEGVPGVGVPGVGVPGVGVPGVGVPGEGVPGVGVPGVGVPGVGVPGVGVPGEGVPGVGVPGVGVPGVGVPGVGVPGEGVPGVGVPGVGVPGVGVPGVGVPGEGVPGVGVPGVGVPGVGVPGVGVPGEGVPGVGVPGVGVPGVGVPGVGVPGEGVPGVGVPGVGVPGVGVPGVGVPGEGVPGVGVPGVGVGIPGVGIPGVGIPGVGIPGVGIPGVGIPGVGIPGVGIPGVGIPGVGIPGVGIPGVGIPGVGIPGVGIPGVGIPGVGIPGVGIPGVGIPGVGIPGVGIPGVGIPGVGIPGVGIPGVGIPGVGIPGVGIPGVGIPGVGIPGVGIPGVGIPGVGIPGVGIPGVGIPGVGIPGVGIPGVGIPGVGIPGVGIPGVGIPGVGIPGVGIPGVGIPGVGIPGVGIPGVGIPGVGIPGVGIPGVGIPGVGIPGVGIPGVGIPGVGIPGVGIPGVGIPGVGIPGVGIPGVGIPGVGIPGVGIPGVGIPGVGAGAGSGAGAGSGAGAGSGAGAGSGAGAGSGVGAGAGSGAGAGSGAGAGSGAGAGSGAGAGSVPGVGVPGVGVPGEGVPGVGVPGVGVPGVGVPGVGVPGEGVPGVGVPGVGVPGVGVPGVGVPGEGVPGVGVPGVGVPGVGVPGVGVPGEGVPGVGVPGVGVPGVGVPGVGVPGEGVPGVGVPGVGVPGVGVPGVGVPGEGVPGVGVPGVGVPGVGVPGVGVPGEGVPGVGVPGVGVPGVGVPGVGVPGEGVPGVGVPGVGVPGVGVPGVGVPGEGVPGVGVPGVGVPGVGVPGVGVPGEGVPGVGVPGVGVGIPGVGIPGVGIPGVGIPGVGIPGVGIPGVGIPGVGIPGVGIPGVGIPGVGIPGVGIPGVGIPGVGIPGVGIPGVGIPGVGIPGVGIPGVGIPGVGIPGVGIPGVGIPGVGIPGVGIPGVGIPGVGIPGVGIPGVGIPGVGIPGVGIPGVGIPGVGIPGVGIPGVGIPGVGIPGVGIPGVGIPGVGIPGVGIPGVGIPGVGIPGVGIPGVGIPGVGIPGVGIPGVGIPGVGIPGVGIPGVGIPGVGIPGVGIPGVGIPGVGIPGVGIPGVGIPGVGIPGVGIPGVGIPGVGIPGVGIPGVGAGAGSGAGAGSGAGAGSGAGAGSGAGAGSGVGAGAGSGAGAGSGAGAGSGAGAGSGAGAGSVPGIGVPGIGVPGIGVPGIGVPGIGAVTGRGDSPASSVPGIGVPGIGVPGIGVPGIGVPGIGAVTGRGDSPASSVPGIGVPGIGVPGIGVPGIGVPGIGAVTGRGDSPASSVPGIGVPGIGVPGIGVPGIGVPGIGAVTGRGDSPASSVPGIGVPGIGVPGIGVPGIGVPGIGAVTGRGDSPASSVPGIGVPGIGVPGIGVPGIGVPGIGAVTGRGDSPASSV

SEQ ID NO: 17 - protein, 4 aa, Artificial Sequence
  DGEA domain
DGEA

SEQ ID NO: 18 - protein, 5 aa, Artificial Sequence
  YIGSR domain
YIGSR

SEQ ID NO: 19 - protein, 9 aa, Artificial Sequence
  QAASIKVAV domain
QAASIKVAV

SEQ ID NO: 20 - protein, 6 aa, Artificial Sequence
  Monomer A
MESLLP

SEQ ID NO: 21 - DNA, 3987 bp, Artificial Sequence
  Nucleotide sequence of the biopolymer 1
atggaatccctgctgccggtaccaggtgttggtgttccgggtgttggcgtgccgggcgaaggcgtgccgggtgttggtgttccgggtgtaggggtaccaggtgttggtgttccgggtgttggcgtgccgggcgaaggcgtgccgggtgttggtgttccgggtgtaggggtaccaggtgttggtgttccgggtgttggcgtgccgggcgaaggcgtgccgggtgttggtgttccgggtgtaggggtaccaggtgttggtgttccgggtgttggcgtgccgggcgaaggcgtgccgggtgttggtgttccgggtgtaggggtaccaggtgttggtgttccgggtgttggcgtgccgggcgaaggcgtgccgggtgttggtgttccgggtgtaggggtaccaggtgttggtgttccgggtgttggcgtgccgggcgaaggcgtgccgggtgttggtgttccgggtgtaggggtaccaggtgttggtgttccgggtgttggcgtgccgggcgaaggcgtgccgggtgttggtgttccgggtgtaggggtaccaggtgttggtgttccgggtgttggcgtgccgggcgaaggcgtgccgggtgttggtgttccgggtgtaggggtaccaggtgttggtgttccgggtgttggcgtgccgggcgaaggcgtgccgggtgttggtgttccgggtgtaggggtaccaggtgttggtgttccgggtgttggcgtgccgggcgaaggcgtgccgggtgttggtgttccgggtgtaggggtaggtatcccgggcgttggtatcccgggcgtgggtattccgggcgttggtatcccgggcgtaggtatcccaggcgttggtatcccgggcgtgggtatcccgggcgttggtattccgggcgtgggtatcccgggcgttggtatccctggtgtaggtatcccgggcgttggtatcccgggcgtgggtattccgggcgttggtatcccgggcgtaggtatcccaggcgttggtatcccgggcgtgggtatcccgggcgttggtattccgggcgtgggtatcccgggcgttggtatccctggtgtaggtatcccgggcgttggtatcccgggcgtgggtattccgggcgttggtatcccgggcgtaggtatcccaggcgttggtatcccgggcgtgggtatcccgggcgttggtattccgggcgtgggtatcccgggcgttggtatccctggtgtaggtatcccgggcgttggtatcccgggcgtgggtattccgggcgttggtatcccgggcgtaggtatcccaggcgttggtatcccgggcgtgggtatcccgggcgttggtattccgggcgtgggtatcccgggcgttggtatccctggtgtaggtatcccgggcgttggtatcccgggcgtgggtattccgggcgttggtatcccgggcgtaggtatcccaggcgttggtatcccgggcgtgggtatcccgggcgttggtattccgggcgtgggtatcccgggcgttggtatccctggtgtaggtatcccgggcgttggtatcccgggcgtgggtattccgggcgttggtatcccgggcgtaggtatcccaggcgttggtatcccgggcgtgggtatcccgggcgttggtattccgggcgtgggtatcccgggcgttggtatccctggtgtaccaggtgttggtgttccgggtgttggcgtgccgggcgaaggcgtgccgggtgttggtgttccgggtgtaggggtaccaggtgttggtgttccgggtgttggcgtgccgggcgaaggcgtgccgggtgttggtgttccgggtgtaggggtaccaggtgttggtgttccgggtgttggcgtgccgggcgaaggcgtgccgggtgttggtgttccgggtgtaggggtaccaggtgttggtgttccgggtgttggcgtgccgggcgaaggcgtgccgggtgttggtgttccgggtgtaggggtaccaggtgttggtgttccgggtgttggcgtgccgggcgaaggcgtgccgggtgttggtgttccgggtgtaggggtaccaggtgttggtgttccgggtgttggcgtgccgggcgaaggcgtgccgggtgttggtgttccgggtgtaggggtaccaggtgttggtgttccgggtgttggcgtgccgggcgaaggcgtgccgggtgttggtgttccgggtgtaggggtaccaggtgttggtgttccgggtgttggcgtgccgggcgaaggcgtgccgggtgttggtgttccgggtgtaggggtaccaggtgttggtgttccgggtgttggcgtgccgggcgaaggcgtgccgggtgttggtgttccgggtgtaggggtaccaggtgttggtgttccgggtgttggcgtgccgggcgaaggcgtgccgggtgttggtgttccgggtgtaggggtaggtatcccgggcgttggtatcccgggcgtgggtattccgggcgttggtatcccgggcgtaggtatcccaggcgttggtatcccgggcgtgggtatcccgggcgttggtattccgggcgtgggtatcccgggcgttggtatccctggtgtaggtatcccgggcgttggtatcccgggcgtgggtattccgggcgttggtatcccgggcgtaggtatcccaggcgttggtatcccgggcgtgggtatcccgggcgttggtattccgggcgtgggtatcccgggcgttggtatccctggtgtaggtatcccgggcgttggtatcccgggcgtgggtattccgggcgttggtatcccgggcgtaggtatcccaggcgttggtatcccgggcgtgggtatcccgggcgttggtattccgggcgtgggtatcccgggcgttggtatccctggtgtaggtatcccgggcgttggtatcccgggcgtgggtattccgggcgttggtatcccgggcgtaggtatcccaggcgttggtatcccgggcgtgggtatcccgggcgttggtattccgggcgtgggtatcccgggcgttggtatccctggtgtaggtatcccgggcgttggtatcccgggcgtgggtattccgggcgttggtatcccgggcgtaggtatcccaggcgttggtatcccgggcgtgggtatcccgggcgttggtattccgggcgtgggtatcccgggcgttggtatccctggtgtaggtatcccgggcgttggtatcccgggcgtgggtattccgggcgttggtatcccgggcgtaggtatcccaggcgttggtatcccgggcgtgggtatcccgggcgttggtattccgggcgtgggtatcccgggcgttggtatccctggtgtaccaggcatcggtgtgccgggcatcggtgttccgggcattggtgtgccgggcatcggtgttccaggcattggtgcagtgaccggtcgtggcgactctcctgcgtccagcgtaccaggcatcggtgtgccgggcatcggtgttccgggcattggtgtgccgggcatcggtgttccaggcattggtgcagtgaccggtcgtggcgactctcctgcgtccagcgtaccaggcatcggtgtgccgggcatcggtgttccgggcattggtgtgccgggcatcggtgttccaggcattggtgcagtgaccggtcgtggcgactctcctgcgtccagcgtaccaggcatcggtgtgccgggcatcggtgttccgggcattggtgtgccgggcatcggtgttccaggcattggtgcagtgaccggtcgtggcgactctcctgcgtccagcgtaccaggcatcggtgtgccgggcatcggtgttccgggcattggtgtgccgggcatcggtgttccaggcattggtgcagtgaccggtcgtggcgactctcctgcgtccagcgtaccaggcatcggtgtgccgggcatcggtgttccgggcattggtgtgccgggcatcggtgttccaggcattggtgcagtgaccggtcgtggcgactctcctgcgtccagcgta

SEQ ID NO: 22 - DNA, 3705 bp, Artificial Sequence
  Nucleotide sequence of the biopolymer 2
atggaatccctgctgccggtaccaggtgttggtgttccgggtgttggcgtgccgggcgaaggcgtgccgggtgttggtgttccgggtgtaggggtaccaggtgttggtgttccgggtgttggcgtgccgggcgaaggcgtgccgggtgttggtgttccgggtgtaggggtaccaggtgttggtgttccgggtgttggcgtgccgggcgaaggcgtgccgggtgttggtgttccgggtgtaggggtaccaggtgttggtgttccgggtgttggcgtgccgggcgaaggcgtgccgggtgttggtgttccgggtgtaggggtaccaggtgttggtgttccgggtgttggcgtgccgggcgaaggcgtgccgggtgttggtgttccgggtgtaggggtaccaggtgttggtgttccgggtgttggcgtgccgggcgaaggcgtgccgggtgttggtgttccgggtgtaggggtaccaggtgttggtgttccgggtgttggcgtgccgggcgaaggcgtgccgggtgttggtgttccgggtgtaggggtaccaggtgttggtgttccgggtgttggcgtgccgggcgaaggcgtgccgggtgttggtgttccgggtgtaggggtaccaggtgttggtgttccgggtgttggcgtgccgggcgaaggcgtgccgggtgttggtgttccgggtgtaggggtaccaggtgttggtgttccgggtgttggcgtgccgggcgaaggcgtgccgggtgttggtgttccgggtgtaggggtaggtatcccgggcgttggtatcccgggcgtgggtattccgggcgttggtatcccgggcgtaggtatcccaggcgttggtatcccgggcgtgggtatcccgggcgttggtattccgggcgtgggtatcccgggcgttggtatccctggtgtaggtatcccgggcgttggtatcccgggcgtgggtattccgggcgttggtatcccgggcgtaggtatcccaggcgttggtatcccgggcgtgggtatcccgggcgttggtattccgggcgtgggtatcccgggcgttggtatccctggtgtaggtatcccgggcgttggtatcccgggcgtgggtattccgggcgttggtatcccgggcgtaggtatcccaggcgttggtatcccgggcgtgggtatcccgggcgttggtattccgggcgtgggtatcccgggcgttggtatccctggtgtaggtatcccgggcgttggtatcccgggcgtgggtattccgggcgttggtatcccgggcgtaggtatcccaggcgttggtatcccgggcgtgggtatcccgggcgttggtattccgggcgtgggtatcccgggcgttggtatccctggtgtaggtatcccgggcgttggtatcccgggcgtgggtattccgggcgttggtatcccgggcgtaggtatcccaggcgttggtatcccgggcgtgggtatcccgggcgttggtattccgggcgtgggtatcccgggcgttggtatccctggtgtaggtatcccgggcgttggtatcccgggcgtgggtattccgggcgttggtatcccgggcgtaggtatcccaggcgttggtatcccgggcgtgggtatcccgggcgttggtattccgggcgtgggtatcccgggcgttggtatccctggtgtaggtgcaggcgcgggttccggcgctggtgccggctctggtgcaggcgcgggtagcggcgctggtgcaggctccggtgcgggcgctggttctggcgtaggtgcaggcgcgggttccggcgctggtgccggctctggtgcaggcgcgggtagcggcgctggtgcaggctccggtgcgggcgctggttctggcgtaccaggtgttggtgttccgggtgttggcgtgccgggcgaaggcgtgccgggtgttggtgttccgggtgtaggggtaccaggtgttggtgttccgggtgttggcgtgccgggcgaaggcgtgccgggtgttggtgttccgggtgtaggggtaccaggtgttggtgttccgggtgttggcgtgccgggcgaaggcgtgccgggtgttggtgttccgggtgtaggggtaccaggtgttggtgttccgggtgttggcgtgccgggcgaaggcgtgccgggtgttggtgttccgggtgtaggggtaccaggtgttggtgttccgggtgttggcgtgccgggcgaaggcgtgccgggtgttggtgttccgggtgtaggggtaccaggtgttggtgttccgggtgttggcgtgccgggcgaaggcgtgccgggtgttggtgttccgggtgtaggggtaccaggtgttggtgttccgggtgttggcgtgccgggcgaaggcgtgccgggtgttggtgttccgggtgtaggggtaccaggtgttggtgttccgggtgttggcgtgccgggcgaaggcgtgccgggtgttggtgttccgggtgtaggggtaccaggtgttggtgttccgggtgttggcgtgccgggcgaaggcgtgccgggtgttggtgttccgggtgtaggggtaccaggtgttggtgttccgggtgttggcgtgccgggcgaaggcgtgccgggtgttggtgttccgggtgtaggggtaggtatcccgggcgttggtatcccgggcgtgggtattccgggcgttggtatcccgggcgtaggtatcccaggcgttggtatcccgggcgtgggtatcccgggcgttggtattccgggcgtgggtatcccgggcgttggtatccctggtgtaggtatcccgggcgttggtatcccgggcgtgggtattccgggcgttggtatcccgggcgtaggtatcccaggcgttggtatcccgggcgtgggtatcccgggcgttggtattccgggcgtgggtatcccgggcgttggtatccctggtgtaggtatcccgggcgttggtatcccgggcgtgggtattccgggcgttggtatcccgggcgtaggtatcccaggcgttggtatcccgggcgtgggtatcccgggcgttggtattccgggcgtgggtatcccgggcgttggtatccctggtgtaggtatcccgggcgttggtatcccgggcgtgggtattccgggcgttggtatcccgggcgtaggtatcccaggcgttggtatcccgggcgtgggtatcccgggcgttggtattccgggcgtgggtatcccgggcgttggtatccctggtgtaggtatcccgggcgttggtatcccgggcgtgggtattccgggcgttggtatcccgggcgtaggtatcccaggcgttggtatcccgggcgtgggtatcccgggcgttggtattccgggcgtgggtatcccgggcgttggtatccctggtgtaggtatcccgggcgttggtatcccgggcgtgggtattccgggcgttggtatcccgggcgtaggtatcccaggcgttggtatcccgggcgtgggtatcccgggcgttggtattccgggcgtgggtatcccgggcgttggtatccctggtgtaggtgcaggcgcgggttccggcgctggtgccggctctggtgcaggcgcgggtagcggcgctggtgcaggctccggtgcgggcgctggttctggcgtaggtgcaggcgcgggttccggcgctggtgccggctctggtgcaggcgcgggtagcggcgctggtgcaggctccggtgcgggcgctggttctggcgta

SEQ ID NO: 23 - DNA, 3639 bp, Artificial Sequence
  Nucleotide sequence of the biopolymer 3
atggaatccctgctgccggtaccaggtgttggtgttccgggtgttggcgtgccgggcgaaggcgtgccgggtgttggtgttccgggtgtaggggtaccaggtgttggtgttccgggtgttggcgtgccgggcgaaggcgtgccgggtgttggtgttccgggtgtaggggtaccaggtgttggtgttccgggtgttggcgtgccgggcgaaggcgtgccgggtgttggtgttccgggtgtaggggtaccaggtgttggtgttccgggtgttggcgtgccgggcgaaggcgtgccgggtgttggtgttccgggtgtaggggtaccaggtgttggtgttccgggtgttggcgtgccgggcgaaggcgtgccgggtgttggtgttccgggtgtaggggtaccaggtgttggtgttccgggtgttggcgtgccgggcgaaggcgtgccgggtgttggtgttccgggtgtaggggtaccaggtgttggtgttccgggtgttggcgtgccgggcgaaggcgtgccgggtgttggtgttccgggtgtaggggtaccaggtgttggtgttccgggtgttggcgtgccgggcgaaggcgtgccgggtgttggtgttccgggtgtaggggtaccaggtgttggtgttccgggtgttggcgtgccgggcgaaggcgtgccgggtgttggtgttccgggtgtaggggtaccaggtgttggtgttccgggtgttggcgtgccgggcgaaggcgtgccgggtgttggtgttccgggtgtaggggtaggtatcccgggcgttggtatcccgggcgtgggtattccgggcgttggtatcccgggcgtaggtatcccaggcgttggtatcccgggcgtgggtatcccgggcgttggtattccgggcgtgggtatcccgggcgttggtatccctggtgtaggtatcccgggcgttggtatcccgggcgtgggtattccgggcgttggtatcccgggcgtaggtatcccaggcgttggtatcccgggcgtgggtatcccgggcgttggtattccgggcgtgggtatcccgggcgttggtatccctggtgtaggtatcccgggcgttggtatcccgggcgtgggtattccgggcgttggtatcccgggcgtaggtatcccaggcgttggtatcccgggcgtgggtatcccgggcgttggtattccgggcgtgggtatcccgggcgttggtatccctggtgtaggtatcccgggcgttggtatcccgggcgtgggtattccgggcgttggtatcccgggcgtaggtatcccaggcgttggtatcccgggcgtgggtatcccgggcgttggtattccgggcgtgggtatcccgggcgttggtatccctggtgtaggtatcccgggcgttggtatcccgggcgtgggtattccgggcgttggtatcccgggcgtaggtatcccaggcgttggtatcccgggcgtgggtatcccgggcgttggtattccgggcgtgggtatcccgggcgttggtatccctggtgtaggtatcccgggcgttggtatcccgggcgtgggtattccgggcgttggtatcccgggcgtaggtatcccaggcgttggtatcccgggcgtgggtatcccgggcgttggtattccgggcgtgggtatcccgggcgttggtatccctggtgtaggcggtggtggtggcaaagaaaaccagattgcgattcgtgccagctttctggaaaaagaaaacagcgcactgcgtcaggaagttgcagacctgcgtaaagaactgggcaaatgcaaaaacattctggcgaaatatgaagcgggtggtggcggtggtgtaccaggtgttggtgttccgggtgttggcgtgccgggcgaaggcgtgccgggtgttggtgttccgggtgtaggggtaccaggtgttggtgttccgggtgttggcgtgccgggcgaaggcgtgccgggtgttggtgttccgggtgtaggggtaccaggtgttggtgttccgggtgttggcgtgccgggcgaaggcgtgccgggtgttggtgttccgggtgtaggggtaccaggtgttggtgttccgggtgttggcgtgccgggcgaaggcgtgccgggtgttggtgttccgggtgtaggggtaccaggtgttggtgttccgggtgttggcgtgccgggcgaaggcgtgccgggtgttggtgttccgggtgtaggggtaccaggtgttggtgttccgggtgttggcgtgccgggcgaaggcgtgccgggtgttggtgttccgggtgtaggggtaccaggtgttggtgttccgggtgttggcgtgccgggcgaaggcgtgccgggtgttggtgttccgggtgtaggggtaccaggtgttggtgttccgggtgttggcgtgccgggcgaaggcgtgccgggtgttggtgttccgggtgtaggggtaccaggtgttggtgttccgggtgttggcgtgccgggcgaaggcgtgccgggtgttggtgttccgggtgtaggggtaccaggtgttggtgttccgggtgttggcgtgccgggcgaaggcgtgccgggtgttggtgttccgggtgtaggggtaggtatcccgggcgttggtatcccgggcgtgggtattccgggcgttggtatcccgggcgtaggtatcccaggcgttggtatcccgggcgtgggtatcccgggcgttggtattccgggcgtgggtatcccgggcgttggtatccctggtgtaggtatcccgggcgttggtatcccgggcgtgggtattccgggcgttggtatcccgggcgtaggtatcccaggcgttggtatcccgggcgtgggtatcccgggcgttggtattccgggcgtgggtatcccgggcgttggtatccctggtgtaggtatcccgggcgttggtatcccgggcgtgggtattccgggcgttggtatcccgggcgtaggtatcccaggcgttggtatcccgggcgtgggtatcccgggcgttggtattccgggcgtgggtatcccgggcgttggtatccctggtgtaggtatcccgggcgttggtatcccgggcgtgggtattccgggcgttggtatcccgggcgtaggtatcccaggcgttggtatcccgggcgtgggtatcccgggcgttggtattccgggcgtgggtatcccgggcgttggtatccctggtgtaggtatcccgggcgttggtatcccgggcgtgggtattccgggcgttggtatcccgggcgtaggtatcccaggcgttggtatcccgggcgtgggtatcccgggcgttggtattccgggcgtgggtatcccgggcgttggtatccctggtgtaggtatcccgggcgttggtatcccgggcgtgggtattccgggcgttggtatcccgggcgtaggtatcccaggcgttggtatcccgggcgtgggtatcccgggcgttggtattccgggcgtgggtatcccgggcgttggtatccctggtgtaggcggtggtggtggcaaagaaaaccagattgcgattcgtgccagctttctggaaaaagaaaacagcgcactgcgtcaggaagttgcagacctgcgtaaagaactgggcaaatgcaaaaacattctggcgaaatatgaagcgggtggtggcggtggtgta

SEQ ID NO: 24 - DNA, 4305 bp, Artificial Sequence
  Nucleotide sequence of the biopolymer 4
atggaatccctgctgccggtaccaggtgttggtgttccgggtgttggcgtgccgggcgaaggcgtgccgggtgttggtgttccgggtgtaggggtaccaggtgttggtgttccgggtgttggcgtgccgggcgaaggcgtgccgggtgttggtgttccgggtgtaggggtaccaggtgttggtgttccgggtgttggcgtgccgggcgaaggcgtgccgggtgttggtgttccgggtgtaggggtaccaggtgttggtgttccgggtgttggcgtgccgggcgaaggcgtgccgggtgttggtgttccgggtgtaggggtaccaggtgttggtgttccgggtgttggcgtgccgggcgaaggcgtgccgggtgttggtgttccgggtgtaggggtaccaggtgttggtgttccgggtgttggcgtgccgggcgaaggcgtgccgggtgttggtgttccgggtgtaggggtaccaggtgttggtgttccgggtgttggcgtgccgggcgaaggcgtgccgggtgttggtgttccgggtgtaggggtaccaggtgttggtgttccgggtgttggcgtgccgggcgaaggcgtgccgggtgttggtgttccgggtgtaggggtaccaggtgttggtgttccgggtgttggcgtgccgggcgaaggcgtgccgggtgttggtgttccgggtgtaggggtaccaggtgttggtgttccgggtgttggcgtgccgggcgaaggcgtgccgggtgttggtgttccgggtgtaggggtaggtatcccgggcgttggtatcccgggcgtgggtattccgggcgttggtatcccgggcgtaggtatcccaggcgttggtatcccgggcgtgggtatcccgggcgttggtattccgggcgtgggtatcccgggcgttggtatccctggtgtaggtatcccgggcgttggtatcccgggcgtgggtattccgggcgttggtatcccgggcgtaggtatcccaggcgttggtatcccgggcgtgggtatcccgggcgttggtattccgggcgtgggtatcccgggcgttggtatccctggtgtaggtatcccgggcgttggtatcccgggcgtgggtattccgggcgttggtatcccgggcgtaggtatcccaggcgttggtatcccgggcgtgggtatcccgggcgttggtattccgggcgtgggtatcccgggcgttggtatccctggtgtaggtatcccgggcgttggtatcccgggcgtgggtattccgggcgttggtatcccgggcgtaggtatcccaggcgttggtatcccgggcgtgggtatcccgggcgttggtattccgggcgtgggtatcccgggcgttggtatccctggtgtaggtatcccgggcgttggtatcccgggcgtgggtattccgggcgttggtatcccgggcgtaggtatcccaggcgttggtatcccgggcgtgggtatcccgggcgttggtattccgggcgtgggtatcccgggcgttggtatccctggtgtaggtatcccgggcgttggtatcccgggcgtgggtattccgggcgttggtatcccgggcgtaggtatcccaggcgttggtatcccgggcgtgggtatcccgggcgttggtattccgggcgtgggtatcccgggcgttggtatccctggtgtaggcggtggtggtggcaaagaaaaccagattgcgattcgtgccagctttctggaaaaagaaaacagcgcactgcgtcaggaagttgcagacctgcgtaaagaactgggcaaatgcaaaaacattctggcgaaatatgaagcgggtggtggcggtggtgtaccaggtgttggtgttccgggtgttggcgtgccgggcgaaggcgtgccgggtgttggtgttccgggtgtaggggtaccaggtgttggtgttccgggtgttggcgtgccgggcgaaggcgtgccgggtgttggtgttccgggtgtaggggtaccaggtgttggtgttccgggtgttggcgtgccgggcgaaggcgtgccgggtgttggtgttccgggtgtaggggtaccaggtgttggtgttccgggtgttggcgtgccgggcgaaggcgtgccgggtgttggtgttccgggtgtaggggtaccaggtgttggtgttccgggtgttggcgtgccgggcgaaggcgtgccgggtgttggtgttccgggtgtaggggtaccaggtgttggtgttccgggtgttggcgtgccgggcgaaggcgtgccgggtgttggtgttccgggtgtaggggtaccaggtgttggtgttccgggtgttggcgtgccgggcgaaggcgtgccgggtgttggtgttccgggtgtaggggtaccaggtgttggtgttccgggtgttggcgtgccgggcgaaggcgtgccgggtgttggtgttccgggtgtaggggtaccaggtgttggtgttccgggtgttggcgtgccgggcgaaggcgtgccgggtgttggtgttccgggtgtaggggtaccaggtgttggtgttccgggtgttggcgtgccgggcgaaggcgtgccgggtgttggtgttccgggtgtaggggtaggtatcccgggcgttggtatcccgggcgtgggtattccgggcgttggtatcccgggcgtaggtatcccaggcgttggtatcccgggcgtgggtatcccgggcgttggtattccgggcgtgggtatcccgggcgttggtatccctggtgtaggtatcccgggcgttggtatcccgggcgtgggtattccgggcgttggtatcccgggcgtaggtatcccaggcgttggtatcccgggcgtgggtatcccgggcgttggtattccgggcgtgggtatcccgggcgttggtatccctggtgtaggtatcccgggcgttggtatcccgggcgtgggtattccgggcgttggtatcccgggcgtaggtatcccaggcgttggtatcccgggcgtgggtatcccgggcgttggtattccgggcgtgggtatcccgggcgttggtatccctggtgtaggtatcccgggcgttggtatcccgggcgtgggtattccgggcgttggtatcccgggcgtaggtatcccaggcgttggtatcccgggcgtgggtatcccgggcgttggtattccgggcgtgggtatcccgggcgttggtatccctggtgtaggtatcccgggcgttggtatcccgggcgtgggtattccgggcgttggtatcccgggcgtaggtatcccaggcgttggtatcccgggcgtgggtatcccgggcgttggtattccgggcgtgggtatcccgggcgttggtatccctggtgtaggtatcccgggcgttggtatcccgggcgtgggtattccgggcgttggtatcccgggcgtaggtatcccaggcgttggtatcccgggcgtgggtatcccgggcgttggtattccgggcgtgggtatcccgggcgttggtatccctggtgtaggcggtggtggtggcaaagaaaaccagattgcgattcgtgccagctttctggaaaaagaaaacagcgcactgcgtcaggaagttgcagacctgcgtaaagaactgggcaaatgcaaaaacattctggcgaaatatgaagcgggtggtggcggtggtgtaccaggcatcggtgtgccgggcatcggtgttccgggcattggtgtgccgggcatcggtgttccaggcattggtgcagtgaccggtcgtggcgactctcctgcgtccagcgtaccaggcatcggtgtgccgggcatcggtgttccgggcattggtgtgccgggcatcggtgttccaggcattggtgcagtgaccggtcgtggcgactctcctgcgtccagcgtaccaggcatcggtgtgccgggcatcggtgttccgggcattggtgtgccgggcatcggtgttccaggcattggtgcagtgaccggtcgtggcgactctcctgcgtccagcgtaccaggcatcggtgtgccgggcatcggtgttccgggcattggtgtgccgggcatcggtgttccaggcattggtgcagtgaccggtcgtggcgactctcctgcgtccagcgtaccaggcatcggtgtgccgggcatcggtgttccgggcattggtgtgccgggcatcggtgttccaggcattggtgcagtgaccggtcgtggcgactctcctgcgtccagcgtaccaggcatcggtgtgccgggcatcggtgttccgggcattggtgtgccgggcatcggtgttccaggcattggtgcagtgaccggtcgtggcgactctcctgcgtccagcgta

SEQ ID NO: 25 - DNA, 4371 bp, Artificial Sequence
  Nucleotide sequence of the biopolymer 5
atggaatccctgctgccggtaccaggtgttggtgttccgggtgttggcgtgccgggcgaaggcgtgccgggtgttggtgttccgggtgtaggggtaccaggtgttggtgttccgggtgttggcgtgccgggcgaaggcgtgccgggtgttggtgttccgggtgtaggggtaccaggtgttggtgttccgggtgttggcgtgccgggcgaaggcgtgccgggtgttggtgttccgggtgtaggggtaccaggtgttggtgttccgggtgttggcgtgccgggcgaaggcgtgccgggtgttggtgttccgggtgtaggggtaccaggtgttggtgttccgggtgttggcgtgccgggcgaaggcgtgccgggtgttggtgttccgggtgtaggggtaccaggtgttggtgttccgggtgttggcgtgccgggcgaaggcgtgccgggtgttggtgttccgggtgtaggggtaccaggtgttggtgttccgggtgttggcgtgccgggcgaaggcgtgccgggtgttggtgttccgggtgtaggggtaccaggtgttggtgttccgggtgttggcgtgccgggcgaaggcgtgccgggtgttggtgttccgggtgtaggggtaccaggtgttggtgttccgggtgttggcgtgccgggcgaaggcgtgccgggtgttggtgttccgggtgtaggggtaccaggtgttggtgttccgggtgttggcgtgccgggcgaaggcgtgccgggtgttggtgttccgggtgtaggggtaggtatcccgggcgttggtatcccgggcgtgggtattccgggcgttggtatcccgggcgtaggtatcccaggcgttggtatcccgggcgtgggtatcccgggcgttggtattccgggcgtgggtatcccgggcgttggtatccctggtgtaggtatcccgggcgttggtatcccgggcgtgggtattccgggcgttggtatcccgggcgtaggtatcccaggcgttggtatcccgggcgtgggtatcccgggcgttggtattccgggcgtgggtatcccgggcgttggtatccctggtgtaggtatcccgggcgttggtatcccgggcgtgggtattccgggcgttggtatcccgggcgtaggtatcccaggcgttggtatcccgggcgtgggtatcccgggcgttggtattccgggcgtgggtatcccgggcgttggtatccctggtgtaggtatcccgggcgttggtatcccgggcgtgggtattccgggcgttggtatcccgggcgtaggtatcccaggcgttggtatcccgggcgtgggtatcccgggcgttggtattccgggcgtgggtatcccgggcgttggtatccctggtgtaggtatcccgggcgttggtatcccgggcgtgggtattccgggcgttggtatcccgggcgtaggtatcccaggcgttggtatcccgggcgtgggtatcccgggcgttggtattccgggcgtgggtatcccgggcgttggtatccctggtgtaggtatcccgggcgttggtatcccgggcgtgggtattccgggcgttggtatcccgggcgtaggtatcccaggcgttggtatcccgggcgtgggtatcccgggcgttggtattccgggcgtgggtatcccgggcgttggtatccctggtgtaggtgcaggcgcgggttccggcgctggtgccggctctggtgcaggcgcgggtagcggcgctggtgcaggctccggtgcgggcgctggttctggcgtaggtgcaggcgcgggttccggcgctggtgccggctctggtgcaggcgcgggtagcggcgctggtgcaggctccggtgcgggcgctggttctggcgtaccaggtgttggtgttccgggtgttggcgtgccgggcgaaggcgtgccgggtgttggtgttccgggtgtaggggtaccaggtgttggtgttccgggtgttggcgtgccgggcgaaggcgtgccgggtgttggtgttccgggtgtaggggtaccaggtgttggtgttccgggtgttggcgtgccgggcgaaggcgtgccgggtgttggtgttccgggtgtaggggtaccaggtgttggtgttccgggtgttggcgtgccgggcgaaggcgtgccgggtgttggtgttccgggtgtaggggtaccaggtgttggtgttccgggtgttggcgtgccgggcgaaggcgtgccgggtgttggtgttccgggtgtaggggtaccaggtgttggtgttccgggtgttggcgtgccgggcgaaggcgtgccgggtgttggtgttccgggtgtaggggtaccaggtgttggtgttccgggtgttggcgtgccgggcgaaggcgtgccgggtgttggtgttccgggtgtaggggtaccaggtgttggtgttccgggtgttggcgtgccgggcgaaggcgtgccgggtgttggtgttccgggtgtaggggtaccaggtgttggtgttccgggtgttggcgtgccgggcgaaggcgtgccgggtgttggtgttccgggtgtaggggtaccaggtgttggtgttccgggtgttggcgtgccgggcgaaggcgtgccgggtgttggtgttccgggtgtaggggtaggtatcccgggcgttggtatcccgggcgtgggtattccgggcgttggtatcccgggcgtaggtatcccaggcgttggtatcccgggcgtgggtatcccgggcgttggtattccgggcgtgggtatcccgggcgttggtatccctggtgtaggtatcccgggcgttggtatcccgggcgtgggtattccgggcgttggtatcccgggcgtaggtatcccaggcgttggtatcccgggcgtgggtatcccgggcgttggtattccgggcgtgggtatcccgggcgttggtatccctggtgtaggtatcccgggcgttggtatcccgggcgtgggtattccgggcgttggtatcccgggcgtaggtatcccaggcgttggtatcccgggcgtgggtatcccgggcgttggtattccgggcgtgggtatcccgggcgttggtatccctggtgtaggtatcccgggcgttggtatcccgggcgtgggtattccgggcgttggtatcccgggcgtaggtatcccaggcgttggtatcccgggcgtgggtatcccgggcgttggtattccgggcgtgggtatcccgggcgttggtatccctggtgtaggtatcccgggcgttggtatcccgggcgtgggtattccgggcgttggtatcccgggcgtaggtatcccaggcgttggtatcccgggcgtgggtatcccgggcgttggtattccgggcgtgggtatcccgggcgttggtatccctggtgtaggtatcccgggcgttggtatcccgggcgtgggtattccgggcgttggtatcccgggcgtaggtatcccaggcgttggtatcccgggcgtgggtatcccgggcgttggtattccgggcgtgggtatcccgggcgttggtatccctggtgtaggtgcaggcgcgggttccggcgctggtgccggctctggtgcaggcgcgggtagcggcgctggtgcaggctccggtgcgggcgctggttctggcgtaggtgcaggcgcgggttccggcgctggtgccggctctggtgcaggcgcgggtagcggcgctggtgcaggctccggtgcgggcgctggttctggcgtaccaggcatcggtgtgccgggcatcggtgttccgggcattggtgtgccgggcatcggtgttccaggcattggtgcagtgaccggtcgtggcgactctcctgcgtccagcgtaccaggcatcggtgtgccgggcatcggtgttccgggcattggtgtgccgggcatcggtgttccaggcattggtgcagtgaccggtcgtggcgactctcctgcgtccagcgtaccaggcatcggtgtgccgggcatcggtgttccgggcattggtgtgccgggcatcggtgttccaggcattggtgcagtgaccggtcgtggcgactctcctgcgtccagcgtaccaggcatcggtgtgccgggcatcggtgttccgggcattggtgtgccgggcatcggtgttccaggcattggtgcagtgaccggtcgtggcgactctcctgcgtccagcgtaccaggcatcggtgtgccgggcatcggtgttccgggcattggtgtgccgggcatcggtgttccaggcattggtgcagtgaccggtcgtggcgactctcctgcgtccagcgtaccaggcatcggtgtgccgggcatcggtgttccgggcattggtgtgccgggcatcggtgttccaggcattggtgcagtgaccggtcgtggcgactctcctgcgtccagcgta

SEQ ID NO: 26 - DNA, 4530 bp, Artificial Sequence
  Nucleotide sequence of the biopolymer 6
atggaatccctgctgccggtaggcggtggtggtggcaaagaaaaccagattgcgattcgtgccagctttctggaaaaagaaaacagcgcactgcgtcaggaagttgcagacctgcgtaaagaactgggcaaatgcaaaaacattctggcgaaatatgaagcgggtggtggcggtggtgtaccaggtgttggtgttccgggtgttggcgtgccgggcgaaggcgtgccgggtgttggtgttccgggtgtaggggtaccaggtgttggtgttccgggtgttggcgtgccgggcgaaggcgtgccgggtgttggtgttccgggtgtaggggtaccaggtgttggtgttccgggtgttggcgtgccgggcgaaggcgtgccgggtgttggtgttccgggtgtaggggtaccaggtgttggtgttccgggtgttggcgtgccgggcgaaggcgtgccgggtgttggtgttccgggtgtaggggtaccaggtgttggtgttccgggtgttggcgtgccgggcgaaggcgtgccgggtgttggtgttccgggtgtaggggtaccaggtgttggtgttccgggtgttggcgtgccgggcgaaggcgtgccgggtgttggtgttccgggtgtaggggtaccaggtgttggtgttccgggtgttggcgtgccgggcgaaggcgtgccgggtgttggtgttccgggtgtaggggtaccaggtgttggtgttccgggtgttggcgtgccgggcgaaggcgtgccgggtgttggtgttccgggtgtaggggtaccaggtgttggtgttccgggtgttggcgtgccgggcgaaggcgtgccgggtgttggtgttccgggtgtaggggtaccaggtgttggtgttccgggtgttggcgtgccgggcgaaggcgtgccgggtgttggtgttccgggtgtaggggtaggtatcccgggcgttggtatcccgggcgtgggtattccgggcgttggtatcccgggcgtaggtatcccaggcgttggtatcccgggcgtgggtatcccgggcgttggtattccgggcgtgggtatcccgggcgttggtatccctggtgtaggtatcccgggcgttggtatcccgggcgtgggtattccgggcgttggtatcccgggcgtaggtatcccaggcgttggtatcccgggcgtgggtatcccgggcgttggtattccgggcgtgggtatcccgggcgttggtatccctggtgtaggtatcccgggcgttggtatcccgggcgtgggtattccgggcgttggtatcccgggcgtaggtatcccaggcgttggtatcccgggcgtgggtatcccgggcgttggtattccgggcgtgggtatcccgggcgttggtatccctggtgtaggtatcccgggcgttggtatcccgggcgtgggtattccgggcgttggtatcccgggcgtaggtatcccaggcgttggtatcccgggcgtgggtatcccgggcgttggtattccgggcgtgggtatcccgggcgttggtatccctggtgtaggtatcccgggcgttggtatcccgggcgtgggtattccgggcgttggtatcccgggcgtaggtatcccaggcgttggtatcccgggcgtgggtatcccgggcgttggtattccgggcgtgggtatcccgggcgttggtatccctggtgtaggtatcccgggcgttggtatcccgggcgtgggtattccgggcgttggtatcccgggcgtaggtatcccaggcgttggtatcccgggcgtgggtatcccgggcgttggtattccgggcgtgggtatcccgggcgttggtatccctggtgtaggtgcaggcgcgggttccggcgctggtgccggctctggtgcaggcgcgggtagcggcgctggtgcaggctccggtgcgggcgctggttctggcgtaggtgcaggcgcgggttccggcgctggtgccggctctggtgcaggcgcgggtagcggcgctggtgcaggctccggtgcgggcgctggttctggcgtaccaggtgttggtgttccgggtgttggcgtgccgggcgaaggcgtgccgggtgttggtgttccgggtgtaggggtaccaggtgttggtgttccgggtgttggcgtgccgggcgaaggcgtgccgggtgttggtgttccgggtgtaggggtaccaggtgttggtgttccgggtgttggcgtgccgggcgaaggcgtgccgggtgttggtgttccgggtgtaggggtaccaggtgttggtgttccgggtgttggcgtgccgggcgaaggcgtgccgggtgttggtgttccgggtgtaggggtaccaggtgttggtgttccgggtgttggcgtgccgggcgaaggcgtgccgggtgttggtgttccgggtgtaggggtaccaggtgttggtgttccgggtgttggcgtgccgggcgaaggcgtgccgggtgttggtgttccgggtgtaggggtaccaggtgttggtgttccgggtgttggcgtgccgggcgaaggcgtgccgggtgttggtgttccgggtgtaggggtaccaggtgttggtgttccgggtgttggcgtgccgggcgaaggcgtgccgggtgttggtgttccgggtgtaggggtaccaggtgttggtgttccgggtgttggcgtgccgggcgaaggcgtgccgggtgttggtgttccgggtgtaggggtaccaggtgttggtgttccgggtgttggcgtgccgggcgaaggcgtgccgggtgttggtgttccgggtgtaggggtaggtatcccgggcgttggtatcccgggcgtgggtattccgggcgttggtatcccgggcgtaggtatcccaggcgttggtatcccgggcgtgggtatcccgggcgttggtattccgggcgtgggtatcccgggcgttggtatccctggtgtaggtatcccgggcgttggtatcccgggcgtgggtattccgggcgttggtatcccgggcgtaggtatcccaggcgttggtatcccgggcgtgggtatcccgggcgttggtattccgggcgtgggtatcccgggcgttggtatccctggtgtaggtatcccgggcgttggtatcccgggcgtgggtattccgggcgttggtatcccgggcgtaggtatcccaggcgttggtatcccgggcgtgggtatcccgggcgttggtattccgggcgtgggtatcccgggcgttggtatccctggtgtaggtatcccgggcgttggtatcccgggcgtgggtattccgggcgttggtatcccgggcgtaggtatcccaggcgttggtatcccgggcgtgggtatcccgggcgttggtattccgggcgtgggtatcccgggcgttggtatccctggtgtaggtatcccgggcgttggtatcccgggcgtgggtattccgggcgttggtatcccgggcgtaggtatcccaggcgttggtatcccgggcgtgggtatcccgggcgttggtattccgggcgtgggtatcccgggcgttggtatccctggtgtaggtatcccgggcgttggtatcccgggcgtgggtattccgggcgttggtatcccgggcgtaggtatcccaggcgttggtatcccgggcgtgggtatcccgggcgttggtattccgggcgtgggtatcccgggcgttggtatccctggtgtaggtgcaggcgcgggttccggcgctggtgccggctctggtgcaggcgcgggtagcggcgctggtgcaggctccggtgcgggcgctggttctggcgtaggtgcaggcgcgggttccggcgctggtgccggctctggtgcaggcgcgggtagcggcgctggtgcaggctccggtgcgggcgctggttctggcgtaccaggcatcggtgtgccgggcatcggtgttccgggcattggtgtgccgggcatcggtgttccaggcattggtgcagtgaccggtcgtggcgactctcctgcgtccagcgtaccaggcatcggtgtgccgggcatcggtgttccgggcattggtgtgccgggcatcggtgttccaggcattggtgcagtgaccggtcgtggcgactctcctgcgtccagcgtaccaggcatcggtgtgccgggcatcggtgttccgggcattggtgtgccgggcatcggtgttccaggcattggtgcagtgaccggtcgtggcgactctcctgcgtccagcgtaccaggcatcggtgtgccgggcatcggtgttccgggcattggtgtgccgggcatcggtgttccaggcattggtgcagtgaccggtcgtggcgactctcctgcgtccagcgtaccaggcatcggtgtgccgggcatcggtgttccgggcattggtgtgccgggcatcggtgttccaggcattggtgcagtgaccggtcgtggcgactctcctgcgtccagcgtaccaggcatcggtgtgccgggcatcggtgttccgggcattggtgtgccgggcatcggtgttccaggcattggtgcagtgaccggtcgtggcgactctcctgcgtccagcgta

SEQ ID NO: 27 - protein, 3 aa, Artificial Sequence
  LDT domain
KDP

SEQ ID NO: 28 - protein, 4 aa, Artificial Sequence
  GTAR domain of uPa enzyme
GTAR

SEQ ID NO: 29 - protein, 4 aa, Artificial Sequence
  DRIR domain of uPa enzyme
DRIR